European Patent Specification EP 4 602 064 B1, published May 13, 2026. Title: Method of manufacturing a peptide with a lysine derivative. Applicant: Bachem Holding AG. Application EP PCT/EP2023/077884, filed October 9, 2023. The sequence listing filed with the application follows.

SEQUENCE LISTING (29 sequences)

SEQ ID NO: 1 - protein, 12 aa, synthetic construct
  MOD_RES 1: note = 2-(p-nitrophenylsulfonyl)ethoxycarbonyl-lysine(17-carboxy-heptadecacarbonyl-gamma-Glu-2-[2-(2-aminoethoxy)ethoxyacetyl]-2-[2-(2-aminoethoxy)ethoxyacetyl])
KEFIAWLVRGRG

SEQ ID NO: 2 - protein, 12 aa, synthetic construct
  MOD_RES 1: note = lysine(17-carboxy-heptadecacarbonyl-gamma-Glu-2-[2-(2-aminoethoxy)ethoxyacetyl]-2-[2-(2-aminoethoxy)ethoxyacetyl])
KEFIAWLVRGRG

SEQ ID NO: 3 - protein, 13 aa, synthetic construct
  MOD_RES 1: note = 9-fluorenylmethyloxycarbonyl-alanine
  MOD_RES 2: note = lysine(17-carboxy-heptadecacarbonyl-gamma-Glu-2-[2-(2-aminoethoxy)ethoxyacetyl]-2-[2-(2-aminoethoxy)ethoxyacetyl])
AKEFIAWLVRGRG

SEQ ID NO: 4 - protein, 13 aa, synthetic construct
  MOD_RES 2: note = lysine(17-carboxy-heptadecacarbonyl-gamma-Glu-2-[2-(2-aminoethoxy)ethoxyacetyl]-2-[2-(2-aminoethoxy)ethoxyacetyl])
AKEFIAWLVRGRG

SEQ ID NO: 5 - protein, 31 aa, synthetic construct
  MOD_RES 2: note = Aib
  MOD_RES 20: note = lysine(17-carboxy-heptadecacarbonyl-gamma-Glu-2-[2-(2-aminoethoxy)ethoxyacetyl]-2-[2-(2-aminoethoxy)ethoxyacetyl])
HXEGTFTSDVSSYLEGQAAKEFIAWLVRGRG

SEQ ID NO: 6 - protein, 10 aa, synthetic construct
FIAWLVRGRG

SEQ ID NO: 7 - protein, 11 aa, synthetic construct
EFIAWLVRGRG

SEQ ID NO: 8 - protein, 12 aa, synthetic construct
  MOD_RES 1: note = alpha-azido-lysine(17-carboxy-heptadecacarbonyl-gamma-Glu-2-[2-(2-aminoethoxy)ethoxy-acetyl]-2-[2-(2-aminoethoxy)ethoxyacetyl])
KEFIAWLVRGRG

SEQ ID NO: 9 - protein, 12 aa, synthetic construct
  MOD_RES 1: note = 9-fluorenylmethyloxycarbonyl-lysine(17-carboxy-heptadecacarbonyl-gamma-Glu-2-[2-(2-aminoethoxy)ethoxyacetyl]-2-[2-(2-aminoethoxy)ethoxyacetyl])
KEFIAWLVRGRG

SEQ ID NO: 10 - protein, 12 aa, synthetic construct
  MOD_RES 1: note = 2-(phenylsulfonyl)ethoxycarbonyl-lysine(17-carboxy-heptadecacarbonyl-gamma-Glu-2-[2-(2-aminoethoxy)ethoxyacetyl]-2-[2-(2-aminoethoxy)ethoxyacetyl])
KEFIAWLVRGRG

SEQ ID NO: 11 - protein, 12 aa, synthetic construct
  MOD_RES 1: note = 1,1-dioxobenzo[b]thiophene-2-yl-methyloxycarbonyl-lysine(17-carboxy-heptadecacarbonyl-gamma-Glu-2-[2-(2-aminoethoxy)ethoxyacetyl]-2-[2-(2-aminoethoxy)ethoxyacetyl])
KEFIAWLVRGRG

SEQ ID NO: 12 - protein, 8 aa, synthetic construct
  MOD_RES 1: note = 2-(phenylsulfonyl)ethoxycarbonyl-D-phenylalanine
  MOD_RES 2: note = S-benzyl-L-cysteine
  MOD_RES 4: note = N-formyl-D-tryptophan
  MOD_RES 5: note = L-lysine(phenylsulfonyl)ethoxycarbonyl)
  MOD_RES 7: note = S-benzyl-L-cysteine
  MOD_RES 8: note = L-threonine(2-(phenylsulfonyl)ethoxycarbonyl)2
FCFWKTCT

SEQ ID NO: 13 - protein, 11 aa, synthetic construct
  MOD_RES 1: note = fluorenylmethoxycarbonyl-L-glutamic acid 5-tert-butyl ester
  MOD_RES 5: note = L-tryptophan(tert-butyloxycarbonyl)
  MOD_RES 8: note = L-arginine(2,2,4,6,7-pentamethyl-2,3-dihydrobenzfuran-5-ylsulfonyl)
  MOD_RES 10: note = L-arginine(2,2,4,6,7-pentamethyl-2,3-dihydrobenzfuran-5-ylsulfonyl)
  MOD_RES 11: note = L-glycine-2-chlorotritylamidomethyl resin
EFIAWLVRGRG

SEQ ID NO: 14 - protein, 11 aa, synthetic construct
  MOD_RES 8: note = L-arginine(2,2,4,6,7-pentamethyl-2,3-dihydrobenzfuran-5-ylsulfonyl)
  MOD_RES 10: note = L-arginine(2,2,4,6,7-pentamethyl-2,3-dihydrobenzfuran-5-ylsulfonyl)
  MOD_RES 5: note = L-tryptophan(tert-butyloxycarbonyl)
  MOD_RES 11: note = L-glycine-2-chlorotritylamidomethyl resin
  MOD_RES 1: note = L-glutamic acid(tert-butyl)
EFIAWLVRGRG

SEQ ID NO: 15 - protein, 12 aa, synthetic construct
  MOD_RES 1: note = N-(9-fluorenylmethoxycarbonyl)-lysine(O-tert-butyl-17-carboxy-heptadecacarbonyl-gamma-Glu-2-[2-(2-aminoethoxy)ethoxyacetyl]-2-[2-(2-aminoethoxy)ethoxyacetyl])
  MOD_RES 2: note = L-glutamic acid(tert-butyl)
  MOD_RES 6: note = L-tryptophan(tert-butyloxycarbonyl)
  MOD_RES 9: note = L-arginine(2,2,4,6,7-pentamethyl-2,3-dihydrobenzfuran-5-ylsulfonyl)
  MOD_RES 12: note = L-glycine-2-chlorotritylamidomethyl resin
KEFIAWLVRGRG

SEQ ID NO: 16 - protein, 31 aa, synthetic construct; identical to SEQ ID NO: 5
  MOD_RES 1: note = tert-butyloxycarbonyl-L-histidine(trityl)
  MOD_RES 2: note = Aib
  MOD_RES 3: note = L-glutamic acid(tert-butyl)
  MOD_RES 5: note = L-threonine(O-tert-butyl)
  MOD_RES 7: note = L-threonine(psi(methyl, methyl)pro)
  MOD_RES 8: note = L-serine(tert-O-butyl)
  MOD_RES 9: note = L-aspartic acid(O-3-methyl-pent-3-yl)
  MOD_RES 11: note = L-serine(tert-O-butyl)
  MOD_RES 12: note = L-serine(tert-O-butyl)
  MOD_RES 13: note = L-tyrosine(tert-O-butyl)
  MOD_RES 15: note = L-glutamic acid(tert-butyl)
  MOD_RES 17: note = L-glutamine(trity)
  MOD_RES 20: note = lysine(O-tert-butyl-17-carboxy-heptadecacarbonyl-gamma-Glu-2-[2-(2-aminoethoxy)ethoxyacetyl]-2-[2-(2-aminoethoxy)ethoxyacetyl])
  MOD_RES 25: note = L-tryptophan(tert-butyloxycarbonyl)
  MOD_RES 21: note = L-glutamic acid(tert-butyl)
  MOD_RES 28: note = L-arginine(2,2,4,6,7-pentamethyl-2,3-dihydrobenzfuran-5-ylsulfonyl)
  MOD_RES 30: note = L-arginine(2,2,4,6,7-pentamethyl-2,3-dihydrobenzfuran-5-ylsulfonyl)
  MOD_RES 31: note = L-glycine-2-chlorotritylamidomethyl resin

SEQ ID NO: 17 - protein, 10 aa, synthetic construct
  MOD_RES 4: note = L-tryptophan(tert-butyloxycarbonyl)
  MOD_RES 7: note = L-arginine(2,2,4,6,7-pentamethyl-2,3-dihydrobenzfuran-5-ylsulfonyl)
  MOD_RES 9: note = L-arginine(2,2,4,6,7-pentamethyl-2,3-dihydrobenzfuran-5-ylsulfonyl)
  MOD_RES 10: note = L-glycine-2-chlorotrityl resin
FIAWLVRGRG

SEQ ID NO: 18 - protein, 12 aa, synthetic construct
  MOD_RES 1: note = N3-lysine(O-tert-butyl-17-carboxy-heptadecacarbonyl-gamma-Glu-2-[2-(2-aminoethoxy)ethoxyacetyl]-2-[2-(2-aminoethoxy)ethoxyacetyl]) MOD_RES
  MOD_RES 12: note = L-glycine-2-chlorotrityl resin
  MOD_RES 9: note = L-arginine(2,2,4,6,7-pentamethyl-2,3-dihydrobenzfuran-5-ylsulfonyl)
  MOD_RES 2: note = L-glutamic acid(tert-butyl)
  MOD_RES 6: note = L-tryptophan(tert-butyloxycarbonyl)
  MOD_RES 11: note = L-arginine(2,2,4,6,7-pentamethyl-2,3-dihydrobenzfuran-5-ylsulfonyl)
KEFIAWLVRGRG

SEQ ID NO: 19 - protein, 12 aa, synthetic construct
  MOD_RES 1: note = lysine(O-tert-butyl-17-carboxy-heptadecacarbonyl-gamma-Glu-2-[2-(2-aminoethoxy)ethoxyacetyl]-2-[2-(2-aminoethoxy)ethoxyacetyl])
  MOD_RES 6: note = L-tryptophan(tert-butyloxycarbonyl)
  MOD_RES 2: note = L-glutamic acid(tert-butyl)
  MOD_RES 9: note = L-arginine(2,2,4,6,7-pentamethyl-2,3-dihydrobenzfuran-5-ylsulfonyl)
  MOD_RES 12: note = L-glycine-2-chlorotrityl resin
  MOD_RES 11: note = L-arginine(2,2,4,6,7-pentamethyl-2,3-dihydrobenzfuran-5-ylsulfonyl)
KEFIAWLVRGRG

SEQ ID NO: 20 - protein, 13 aa, synthetic construct
  MOD_RES 1: note = N-(9-fluorenylmethoxycarbonyl)-L-alanine
  MOD_RES 2: note = lysine(O-tert-butyl-17-carboxy-heptadecacarbonyl-gamma-Glu-2-[2-(2-aminoethoxy)ethoxyacetyl]-2-[2-(2-aminoethoxy)ethoxyacetyl])
  MOD_RES 3: note = L-glutamic acid(tert-butyl)
  MOD_RES 7: note = L-tryptophan(tert-butyloxycarbonyl)
  MOD_RES 10: note = L-arginine(2,2,4,6,7-pentamethyl-2,3-dihydrobenzfuran-5-ylsulfonyl)
  MOD_RES 13: note = L-glycine-2-chlorotrityl resin
  MOD_RES 12: note = L-arginine(2,2,4,6,7-pentamethyl-2,3-dihydrobenzfuran-5-ylsulfonyl)
AKEFIAWLVRGRG

SEQ ID NO: 21 - protein, 11 aa, synthetic construct
  MOD_RES 1: note = L-glutamic acid(tert-butyl)
  MOD_RES 5: note = L-tryptophan(tert-butyloxycarbonyl)
  MOD_RES 8: note = L-arginine(2,2,4,6,7-pentamethyl-2,3-dihydrobenzfuran-5-ylsulfonyl)
  MOD_RES 10: note = L-arginine(2,2,4,6,7-pentamethyl-2,3-dihydrobenzfuran-5-ylsulfonyl)
  MOD_RES 11: note = L-glycine-2-chlorotrityl resin
EFIAWLVRGRG

SEQ ID NO: 22 - protein, 12 aa, synthetic construct
  MOD_RES 1: note = N-(9-fluorenylmethoxycarbonyl)-lysine(O-tert-butyl-17-carboxy-heptadecacarbonyl-gamma-Glu-2-[2-(2-aminoethoxy)ethoxyacetyl]-2-[2-(2-aminoethoxy)ethoxyacetyl])
  MOD_RES 2: note = L-glutamic acid(tert-butyl)
  MOD_RES 12: note = L-glycine-2-chlorotrityl resin
  MOD_RES 6: note = L-tryptophan(tert-butyloxycarbonyl)
  MOD_RES 9: note = L-arginine(2,2,4,6,7-pentamethyl-2,3-dihydrobenzfuran-5-ylsulfonyl)
  MOD_RES 11: note = L-arginine(2,2,4,6,7-pentamethyl-2,3-dihydrobenzfuran-5-ylsulfonyl)
KEFIAWLVRGRG

SEQ ID NO: 23 - protein, 12 aa, synthetic construct
  MOD_RES 1: note = 1,1-dioxobenzo[b]thiophen-2-ylmethyloxycarbonyl-lysine(O-tert-butyl-17-carboxy-heptadecacarbonyl-gamma-Glu-2-[2-(2-aminoethoxy)ethoxyacetyl]-2-[2-(2-aminoethoxy)ethoxyacetyl])
  MOD_RES 12: note = L-glycine-2-chlorotrityl resin
  MOD_RES 2: note = L-glutamic acid(tert-butyl)
  MOD_RES 6: note = L-tryptophan(tert-butyloxycarbonyl)
  MOD_RES 9: note = L-arginine(2,2,4,6,7-pentamethyl-2,3-dihydrobenzfuran-5-ylsulfonyl)
  MOD_RES 11: note = L-arginine(2,2,4,6,7-pentamethyl-2,3-dihydrobenzfuran-5-ylsulfonyl)
KEFIAWLVRGRG

SEQ ID NO: 24 - protein, 12 aa, synthetic construct
  MOD_RES 1: note = 2-(phenylsulfonyl)ethoxycarbonyl-lysine(O-tert-butyl-17-carboxy-heptadecacarbonyl-gamma-Glu-2-[2-(2-aminoethoxy)ethoxyacetyl]-2-[2-(2-aminoethoxy)ethoxyacetyl])
  MOD_RES 2: note = L-glutamic acid(tert-butyl)
  MOD_RES 12: note = L-glycine-2-chlorotrityl resin
  MOD_RES 6: note = L-tryptophan(tert-butyloxycarbonyl)
  MOD_RES 9: note = L-arginine(2,2,4,6,7-pentamethyl-2,3-dihydrobenzfuran-5-ylsulfonyl)
  MOD_RES 11: note = L-arginine(2,2,4,6,7-pentamethyl-2,3-dihydrobenzfuran-5-ylsulfonyl)
KEFIAWLVRGRG

SEQ ID NO: 25 - protein, 12 aa, synthetic construct
  MOD_RES 1: note = 2-(p-nitrophenylsulfonyl)ethoxycarbonyl-lysine(O-tert-butyl-17-carboxy-heptadecacarbonyl-gamma-Glu-2-[2-(2-aminoethoxy)ethoxyacetyl]-2-[2-(2-aminoethoxy)ethoxyacetyl])
  MOD_RES 2: note = L-glutamic acid(tert-butyl)
  MOD_RES 6: note = L-tryptophan(tert-butyloxycarbonyl)
  MOD_RES 9: note = L-arginine(2,2,4,6,7-pentamethyl-2,3-dihydrobenzfuran-5-ylsulfonyl)
  MOD_RES 11: note = L-arginine(2,2,4,6,7-pentamethyl-2,3-dihydrobenzfuran-5-ylsulfonyl)
  MOD_RES 12: note = L-glycine-2-chlorotrityl resin
KEFIAWLVRGRG

SEQ ID NO: 26 - protein, 12 aa, synthetic construct
  MOD_RES 1: note = 2-(p-nitrophenylsulfonyl)ethoxycarbonyl-lysine(O-tert-butyl-17-carboxy-heptadecacarbonyl-gamma-Glu-2-[2-(2-aminoethoxy)ethoxyacetyl]-2-[2-(2-aminoethoxy)ethoxyacetyl])
  MOD_RES 2: note = L-glutamic acid(tert-butyl)
  MOD_RES 6: note = L-tryptophan(tert-butyloxycarbonyl)
  MOD_RES 12: note = L-glycine-2-chlorotritylamidomethyl resin
  MOD_RES 9: note = L-arginine(2,2,4,6,7-pentamethyl-2,3-dihydrobenzfuran-5-ylsulfonyl)
  MOD_RES 11: note = L-arginine(2,2,4,6,7-pentamethyl-2,3-dihydrobenzfuran-5-ylsulfonyl)
KEFIAWLVRGRG

SEQ ID NO: 27 - protein, 13 aa, synthetic construct
  MOD_RES 3: note = L-glutamic acid(tert-butyl)
  MOD_RES 10: note = L-arginine(2,2,4,6,7-pentamethyl-2,3-dihydrobenzfuran-5-ylsulfonyl)
  MOD_RES 12: note = L-arginine(2,2,4,6,7-pentamethyl-2,3-dihydrobenzfuran-5-ylsulfonyl)
  MOD_RES 13: note = L-glycine-2-chlorotrityl resin
  MOD_RES 7: note = L-tryptophan(tert-butyloxycarbonyl)
  MOD_RES 7: note = L-tryptophan(tert-butyloxycarbonyl)
  MOD_RES 2: note = lysine(O-tert-butyl-17-carboxy-heptadecacarbonyl-gamma-Glu-2-[2-(2-aminoethoxy)ethoxyacetyl]-2-[2-(2-aminoethoxy)ethoxyacetyl])
AKEFIAWLVRGRG

SEQ ID NO: 28 - protein, 12 aa, synthetic construct
  MOD_RES 1: note = lysine(O-tert-butyl-17-carboxy-heptadecacarbonyl-gamma-Glu-2-[2-(2-aminoethoxy)ethoxyacetyl]-2-[2-(2-aminoethoxy)ethoxyacetyl])
  MOD_RES 2: note = L-glutamic acid(tert-butyl)
  MOD_RES 6: note = L-tryptophan(tert-butyloxycarbonyl)
  MOD_RES 9: note = L-arginine(2,2,4,6,7-pentamethyl-2,3-dihydrobenzfuran-5-ylsulfonyl)
  MOD_RES 11: note = L-arginine(2,2,4,6,7-pentamethyl-2,3-dihydrobenzfuran-5-ylsulfonyl)
  MOD_RES 12: note = L-glycine-2-chlorotritylamidomethyl resin
KEFIAWLVRGRG

SEQ ID NO: 29 - protein, 13 aa, synthetic construct
  MOD_RES 2: note = lysine(O-tert-butyl-17-carboxy-heptadecacarbonyl-gamma-Glu-2-[2-(2-aminoethoxy)ethoxyacetyl]-2-[2-(2-aminoethoxy)ethoxyacetyl])
  MOD_RES 3: note = L-glutamic acid(tert-butyl)
  MOD_RES 7: note = L-tryptophan(tert-butyloxycarbonyl)
  MOD_RES 10: note = L-arginine(2,2,4,6,7-pentamethyl-2,3-dihydrobenzfuran-5-ylsulfonyl)
  LIPID 12: note = L-arginine(2,2,4,6,7-pentamethyl-2,3-dihydrobenzfuran-5-ylsulfonyl)
  MOD_RES 13: note = L-glycine-2-chlorotritylamidomethyl resin
AKEFIAWLVRGRG